European Patent Application EP 4 464 784 A1, published November 20, 2024. Title: SCHWANN CELL-SPECIFIC PROMOTER. Applicant: TOOLGEN INCORPORATED. Application KR PCT/KR2023/000569, filed January 12, 2023. The sequence listing filed with the application follows.

SEQUENCE LISTING (34 sequences)

SEQ ID NO: 1 - DNA, 1082 bp, synthetic construct
  misc_feature 1..1082: note = Rat MPZ promoter
  source 1..1082: mol_type = other DNA
aacacagatggcacatatctactctaaatatatgcagagcttcacaaacgtcatacacatacgtgtgtcacacacgcacacacacacccttccacctctgcccttacctttgctgtcccatctagacattatccctcccatccccttatttcccttatcaaaatggctgctccttcaaggttccaaataacactgcttcctggacctgactcctctttcctctgaacttcctgtgttaagtggtattcctagtgcactgtgccttggtagttgttgagattgccctctgcttctcccttctgcctcctcatctagtgatcttgagcttgtagaaagaactgaattaccattctaatacgagcattctcgaactctccaaatagccaccaagcaggacaataggcagtcttgatcatttaaactgctgcatggcaaaaggaatcgaaggatttcttaacagaagtggggggggggggagatctgggcttcttcctggaagtttcctgatagagaaaatcttctgcctgggtagaatctcccaggatgcagggagatggaaaaagttgttcccagaggactttgtagtctacagtgttgtcgtagccatcggaacaacgagacaccctaatttgggagtgctctgaaagaaacttgcctctaggccctagggctctcaggcaaggaggctaagaaggaatcctttgctgtagccttttggatttaggtttctcagcttatctatccctcagagaagtgtgtctatgtcccttttctgtccctctgcctcaccccaccccaacattccaacctagggtagggggaggtcagtatacacaaagccctctgtgtaaggggtggtatgtgtccccccacccccctacccagagtatacaatgccccttctgctccatgcccctgccaccctccccaccacctctcaattgcacatgccaggctgcaattggtcactggctcaggacagccccctcatgctggggatccaggggattttaagcaggttccagaaaacaccactcagttccttgtcccccgctctctccaccccacagacgctctgggcc

SEQ ID NO: 2 - DNA, 1000 bp, synthetic construct
  misc_feature 1..1000: note = human MPZ promoter
  source 1..1000: mol_type = other DNA
actatgcctggcataaacttcatttattaaagtttattttgtctttaatctctcatataacttagtcttcctgatattgcagctgtgtgtgcccctcttttgtactcccagcattttgttcattactaaaggaagtgtcatggcttattatacttgattgttgatgggtttgtcctctgatcttcccatctccacctccccaaaccaaattttcaactccttgctggaaggacttaatttttattcctctctctattacctgcattctcatactttacatattgctggcacttaatacaattttgtagccttgaaataaattgaaatggacttaaacagcagcatgaagcactgaaggacttcttgacaaacggaaaggtcaggggcttcttgcctggaaatagtccagtggagaaaaacttctgtctgggaagaatcgcacaggatgaagggaggtgcggggaaaaaaactcccataggacttggtcatctcaagaagtctgtaatgcagcccacattagaggagataacaggggatatcctattttcagagttctctgggggaaacctccctctagttcctagggctgtgaggcagcctctctcaggcaaggaggctgaggagaaatccctttttatggcctttaaattgaggttccatatctatccctcagagaagtgtgtctgtgtccctgtttttgtccctctccctcaccaccccccacaacattccagcctggggcagggggaggccagtggacacaaagccctctgtgtatggggtggtatgtgtccccccacccctccacccagactatacaatgccccttctgctccctgcactctgcccccctccccaccacctctcaactgcacatgccaggctgcaattggttactggctgaggacagccccctcatgctggggccctaggggattttaagcaggttccaggaaccccccgttcagttcctggtcccccactttctcaaccccacag

SEQ ID NO: 3 - DNA, 300 bp, synthetic construct
  misc_feature 1..300: note = Schwann cell specific promoter
  source 1..300: mol_type = other DNA
gcctcaccccaccccaacattccaacctagggtagggggaggtcagtatacacaaagccctctgtgtaaggggtggtatgtgtccccccacccccctacccagagtatacaatgccccttctgctccatgcccctgccaccctccccaccacctctcaattgcacatgccaggctgcaattggtcactggctcaggacagccccctcatgctggggatccaggggattttaagcaggttccagaaaacaccactcagttccttgtcccccgctctctccaccccacagacgctctgggcc

SEQ ID NO: 4 - DNA, 200 bp, synthetic construct
  misc_feature 1..200: note = Schwann cell specific promoter
  source 1..200: mol_type = other DNA
cagagtatacaatgccccttctgctccatgcccctgccaccctccccaccacctctcaattgcacatgccaggctgcaattggtcactggctcaggacagccccctcatgctggggatccaggggattttaagcaggttccagaaaacaccactcagttccttgtcccccgctctctccaccccacagacgctctgggcc

SEQ ID NO: 5 - DNA, 300 bp, synthetic construct
  misc_feature 1..300: note = Schwann cell specific promoter
  source 1..300: mol_type = other DNA
gtccctctccctcaccaccccccacaacattccagcctggggcagggggaggccagtggacacaaagccctctgtgtatggggtggtatgtgtccccccacccctccacccagactatacaatgccccttctgctccctgcactctgcccccctccccaccacctctcaactgcacatgccaggctgcaattggttactggctgaggacagccccctcatgctggggccctaggggattttaagcaggttccaggaaccccccgttcagttcctggtcccccactttctcaaccccacag

SEQ ID NO: 6 - DNA, 200 bp, synthetic construct
  misc_feature 1..200: note = Schwann cell specific promoter
  source 1..200: mol_type = other DNA
cccctccacccagactatacaatgccccttctgctccctgcactctgcccccctccccaccacctctcaactgcacatgccaggctgcaattggttactggctgaggacagccccctcatgctggggccctaggggattttaagcaggttccaggaaccccccgttcagttcctggtcccccactttctcaaccccacag

SEQ ID NO: 7 - DNA, 117 bp, synthetic construct
  misc_feature 1..117: note = Intronic enhancer
  source 1..117: mol_type = other DNA
gacaatgagactttgtttggtcgcctcctcctaaagaacagaaaagtctataattgttcctccccagagccagcccacacacatagactgcctgggatgactctccctgtgtgggcg

SEQ ID NO: 8 - DNA, 417 bp, synthetic construct
  misc_feature 1..417: note = Schwann cell specific promoter
  source 1..417: mol_type = other DNA
gacaatgagactttgtttggtcgcctcctcctaaagaacagaaaagtctataattgttcctccccagagccagcccacacacatagactgcctgggatgactctccctgtgtgggcggcctcaccccaccccaacattccaacctagggtagggggaggtcagtatacacaaagccctctgtgtaaggggtggtatgtgtccccccacccccctacccagagtatacaatgccccttctgctccatgcccctgccaccctccccaccacctctcaattgcacatgccaggctgcaattggtcactggctcaggacagccccctcatgctggggatccaggggattttaagcaggttccagaaaacaccactcagttccttgtcccccgctctctccaccccacagacgctctgggcc

SEQ ID NO: 9 - DNA, 317 bp, synthetic construct
  misc_feature 1..317: note = Schwann cell specific promoter
  source 1..317: mol_type = other DNA
gacaatgagactttgtttggtcgcctcctcctaaagaacagaaaagtctataattgttcctccccagagccagcccacacacatagactgcctgggatgactctccctgtgtgggcgcagagtatacaatgccccttctgctccatgcccctgccaccctccccaccacctctcaattgcacatgccaggctgcaattggtcactggctcaggacagccccctcatgctggggatccaggggattttaagcaggttccagaaaacaccactcagttccttgtcccccgctctctccaccccacagacgctctgggcc

SEQ ID NO: 10 - DNA, 123 bp, synthetic construct
  misc_feature 1..123: note = Intronic enhancer
  source 1..123: mol_type = other DNA
gacaatggaactttgtttggttgccacctccccctcctgtagaacaaaaaggtctacagttgcccctccctggggccagcccacacacatagtctctctggaatgaccttccttgtgtgggta

SEQ ID NO: 11 - DNA, 423 bp, synthetic construct
  misc_feature 1..423: note = Schwann cell specific promoter
  source 1..423: mol_type = other DNA
gacaatggaactttgtttggttgccacctccccctcctgtagaacaaaaaggtctacagttgcccctccctggggccagcccacacacatagtctctctggaatgaccttccttgtgtgggtagtccctctccctcaccaccccccacaacattccagcctggggcagggggaggccagtggacacaaagccctctgtgtatggggtggtatgtgtccccccacccctccacccagactatacaatgccccttctgctccctgcactctgcccccctccccaccacctctcaactgcacatgccaggctgcaattggttactggctgaggacagccccctcatgctggggccctaggggattttaagcaggttccaggaaccccccgttcagttcctggtcccccactttctcaaccccacag

SEQ ID NO: 12 - DNA, 323 bp, synthetic construct
  misc_feature 1..323: note = Schwann cell specific promoter
  source 1..323: mol_type = other DNA
gacaatggaactttgtttggttgccacctccccctcctgtagaacaaaaaggtctacagttgcccctccctggggccagcccacacacatagtctctctggaatgaccttccttgtgtgggtacccctccacccagactatacaatgccccttctgctccctgcactctgcccccctccccaccacctctcaactgcacatgccaggctgcaattggttactggctgaggacagccccctcatgctggggccctaggggattttaagcaggttccaggaaccccccgttcagttcctggtcccccactttctcaaccccacag

SEQ ID NO: 13 - DNA, 417 bp, synthetic construct
  misc_feature 1..417: note = Schwann cell specific promoter
  source 1..417: mol_type = other DNA
gcctcaccccaccccaacattccaacctagggtagggggaggtcagtatacacaaagccctctgtgtaaggggtggtatgtgtccccccacccccctacccagagtatacaatgccccttctgctccatgcccctgccaccctccccaccacctctcaattgcacatgccaggctgcaattggtcactggctcaggacagccccctcatgctggggatccaggggattttaagcaggttccagaaaacaccactcagttccttgtcccccgctctctccaccccacagacgctctgggccgacaatgagactttgtttggtcgcctcctcctaaagaacagaaaagtctataattgttcctccccagagccagcccacacacatagactgcctgggatgactctccctgtgtgggcg

SEQ ID NO: 14 - DNA, 317 bp, synthetic construct
  misc_feature 1..317: note = Schwann cell specific promoter
  source 1..317: mol_type = other DNA
cagagtatacaatgccccttctgctccatgcccctgccaccctccccaccacctctcaattgcacatgccaggctgcaattggtcactggctcaggacagccccctcatgctggggatccaggggattttaagcaggttccagaaaacaccactcagttccttgtcccccgctctctccaccccacagacgctctgggccgacaatgagactttgtttggtcgcctcctcctaaagaacagaaaagtctataattgttcctccccagagccagcccacacacatagactgcctgggatgactctccctgtgtgggcg

SEQ ID NO: 15 - DNA, 423 bp, synthetic construct
  misc_feature 1..423: note = Schwann cell specific promoter
  source 1..423: mol_type = other DNA
gtccctctccctcaccaccccccacaacattccagcctggggcagggggaggccagtggacacaaagccctctgtgtatggggtggtatgtgtccccccacccctccacccagactatacaatgccccttctgctccctgcactctgcccccctccccaccacctctcaactgcacatgccaggctgcaattggttactggctgaggacagccccctcatgctggggccctaggggattttaagcaggttccaggaaccccccgttcagttcctggtcccccactttctcaaccccacaggacaatggaactttgtttggttgccacctccccctcctgtagaacaaaaaggtctacagttgcccctccctggggccagcccacacacatagtctctctggaatgaccttccttgtgtgggta

SEQ ID NO: 16 - DNA, 323 bp, synthetic construct
  misc_feature 1..323: note = Schwann cell specific promoter
  source 1..323: mol_type = other DNA
cccctccacccagactatacaatgccccttctgctccctgcactctgcccccctccccaccacctctcaactgcacatgccaggctgcaattggttactggctgaggacagccccctcatgctggggccctaggggattttaagcaggttccaggaaccccccgttcagttcctggtcccccactttctcaaccccacaggacaatggaactttgtttggttgccacctccccctcctgtagaacaaaaaggtctacagttgcccctccctggggccagcccacacacatagtctctctggaatgaccttccttgtgtgggta

SEQ ID NO: 17 - DNA, 104 bp, synthetic construct
  misc_feature 1..104: note = simian virus 40 polyadenylation signal
  source 1..104: mol_type = other DNA
tgctttatttgtaaccattataagctgcaataaacaagttaacaacaacaattgcattcattttatgtttcaggttcagggggagatgtgggaggttttttaaa

SEQ ID NO: 18 - DNA, 92 bp, synthetic construct
  misc_feature 1..92: note = synthetic polyadenylation signal
  source 1..92: mol_type = other DNA
aagaggtaagggtttaagggatggttggttggtggggtattaatgtttaattacctggagcacctgcctgaaatcactttttttcaggttgg

SEQ ID NO: 19 - DNA, 247 bp, synthetic construct
  misc_feature 1..247: note = WPRE3
  source 1..247: mol_type = other DNA
aatcaacctctggattacaaaatttgtgaaagattgactggtattcttaactatgttgctccttttacgctatgtggatacgctgctttaatgcctttgtatcatgctattgcttcccgtatggctttcattttctcctccttgtataaatcctggttagttcttgccacggcggaactcatcgccgcctgccttgcccgctgctggacaggggctcggctgttgggcactgacaattccgtggtgt

SEQ ID NO: 20 - DNA, 592 bp, synthetic construct
  misc_feature 1..592: note = WPRE
  source 1..592: mol_type = other DNA
aatcaacctctggattacaaaatttgtgaaagattgactggtattcttaactatgttgctccttttacgctatgtggatacgctgctttaatgcctttgtatcatgctattgcttcccgtatggctttcattttctcctccttgtataaatcctggttgctgtctctttatgaggagttgtggcccgttgtcaggcaacgtggcgtggtgtgcactgtgtttgctgacgcaacccccactggttggggcattgccaccacctgtcagctcctttccgggactttcgctttccccctccctattgccacggcggaactcatcgccgcctgccttgcccgctgctggacaggggctcggctgttgggcactgacaattccgtggtgttgtcggggaagctgacgtcctttccatggctgctcgcctgtgttgccacctggattctgcgcgggacgtccttctgctacgtcccttcggccctcaatccagcggaccttccttcccgcggcctgctgccggctctgcggcctcttccgcgtcttcgccttcgccctcagacgagtcggatctccctttgggccgcctccccgcctg

SEQ ID NO: 21 - DNA, 92 bp, synthetic construct; identical to SEQ ID NO: 18
  misc_feature 1..92: note = MVM intron
  source 1..92: mol_type = other DNA

SEQ ID NO: 22 - DNA, 23 bp, synthetic construct
  misc_feature 1..23: note = Target Sequence with PAM (5'-3')
  source 1..23: mol_type = other DNA
ggaccagcccctgaataaactgg

SEQ ID NO: 23 - DNA, 25 bp, synthetic construct
  misc_feature 1..25: note = Target Sequence with PAM (5'-3')
  source 1..25: mol_type = other DNA
attcaggggctggtccaatgctggg

SEQ ID NO: 24 - DNA, 20 bp, synthetic construct
  misc_feature 1..20: note = SpCas9 forward primer
  source 1..20: mol_type = other DNA
ggacttctaccccttcctga

SEQ ID NO: 25 - DNA, 19 bp, synthetic construct
  misc_feature 1..19: note = SpCas9 reverse primer
  source 1..19: mol_type = other DNA
gtgatggtctcctcgctct

SEQ ID NO: 26 - DNA, 22 bp, synthetic construct
  misc_feature 1..22: note = hGAPDH forward primer
  source 1..22: mol_type = other DNA
gtctcctctgacttcaacagcg

SEQ ID NO: 27 - DNA, 22 bp, synthetic construct
  misc_feature 1..22: note = hGAPDH reverse primer
  source 1..22: mol_type = other DNA
accaccctgttgctgtagccaa

SEQ ID NO: 28 - DNA, 20 bp, synthetic construct
  misc_feature 1..20: note = rGAPDH forward primer
  source 1..20: mol_type = other DNA
gaaacccatcaccatcttcc

SEQ ID NO: 29 - DNA, 21 bp, synthetic construct
  misc_feature 1..21: note = rGAPDH reverse primer
  source 1..21: mol_type = other DNA
gttcacacccatcacaaacat

SEQ ID NO: 30 - DNA, 21 bp, synthetic construct
  misc_feature 1..21: note = rPMP22 forward primer
  source 1..21: mol_type = other DNA
tccaagttcatttcctgcagg

SEQ ID NO: 31 - DNA, 20 bp, synthetic construct
  misc_feature 1..20: note = rPMP22 reverse primer
  source 1..20: mol_type = other DNA
ccaggctccctgagatgttc

SEQ ID NO: 32 - DNA, 212 bp, synthetic construct
  source 1..212: mol_type = other DNA
  misc_feature 1..212: note = EPS promoter
gggcagagcgcacatcgcccacagtccccgagaagttggggggaggggtcggcaattgatccggtgcctagagaaggtggcgcggggtaaactgggaaagtgatgtcgtgtactggctccgcctttttcccgagggtgggggagaaccgtatataagtgcagtagtcgccgtgaacgttctttttcgcaacgggtttgccgccagaacacag

SEQ ID NO: 33 - DNA, 1431 bp, synthetic construct
  source 1..1431: mol_type = other DNA
  misc_feature 1..1431: note = dtTomato
atggtgagcaagggcgaggaggtcatcaaagagttcatgcgcttcaaggtgcgcatggagggctccatgaacggccacgagttcgagatcgagggcgagggcgagggccgcccctacgagggcacccagaccgccaagctgaaggtgaccaagggcggccccctgcccttcgcctgggacatcctgtccccccagttcatgtacggctccaaggcgtacgtgaagcaccccgccgacatccccgattacaagaagctgtccttccccgagggcttcaagtgggagcgcgtgatgaacttcgaggacggcggtctggtgaccgtgacccaggactcctccctgcaggacggcacgctgatctacaaggtgaagatgcgcggcaccaacttcccccccgacggccccgtaatgcagaagaagaccatgggctgggaggcctccaccgagcgcctgtacccccgcgacggcgtgctgaagggcgagatccaccaggccctgaagctgaaggacggcggccactacctggtggagttcaagaccatctacatggccaagaagcccgtgcaactgcccggctactactacgtggacaccaagctggacatcacctcccacaacgaggactacaccatcgtggaacagtacgagcgctccgagggccgccaccacctgttcctggggcatggcaccggcagcaccggcagcggcagctccggcaccgcctcctccgaggacaacaacatggccgtcatcaaagagttcatgcgcttcaaggtgcgcatggagggctccatgaacggccacgagttcgagatcgagggcgagggcgagggccgcccctacgagggcacccagaccgccaagctgaaggtgaccaagggcggccccctgcccttcgcctgggacatcctgtccccccagttcatgtacggctccaaggcgtacgtgaagcaccccgccgacatccccgattacaagaagctgtccttccccgagggcttcaagtgggagcgcgtgatgaacttcgaggacggcggtctggtgaccgtgacccaggactcctccctgcaggacggcacgctgatctacaaggtgaagatgcgcggcaccaacttcccccccgacggccccgtaatgcagaagaagaccatgggctgggaggcctccaccgagcgcctgtacccccgcgacggcgtgctgaagggcgagatccaccaggccctgaagctgaaggacggcggccactacctggtggagttcaagaccatctacatggccaagaagcccgtgcaactgcccggctactactacgtggacaccaagctggacatcacctcccacaacgaggactacaccatcgtggaacagtacgagcgctccgagggccgccaccacctgttcctgtacggcatggacgagctgtacaagtag

SEQ ID NO: 34 - DNA, 22 bp, synthetic construct
  source 1..22: mol_type = other DNA
  misc_feature 1..22: note = Target Sequence with PAM (5'-3')
gaccagcccctgaataaactgg